European Patent Specification EP 3 500 301 B1, published August 30, 2023. Title: Monovalent Asymmetric Tandem Fab Bispecific Antibodies. Applicant: EPIMAB BIOTHERAPEUTICS, INC. WU, Chengbin. Application PCT/US2017/046875. The sequence listing filed with the application follows.

SEQUENCE LISTING (8 sequences)

SEQ ID NO: 1 - protein, 691 aa, Artificial Sequence
  hybrid immunoglobulin utilizing sequences derived from different organisms
MDMRVPAQLLGLLLLWFPGSRCEIVLTQSPATLSLSPGERATLSCRASQSVSSYLAWYQQKPGQAPRLLIYDASNRATGIPARFSGSGSGTDFTLTISSLEPEDFAVYYCQQRSNWPITFGQGTRLEIKRTVAAPSVFIFPPSDEQLKSGTASVVCLLNNFYPREAKVQWKVDNALQSGNSQESVTEQDSKDSTYSLSSTLTLSKADYEKHKVYACEVTHQGLSSPVTKSFNRGECEVQLLESGGGLVQPGGSLKLSCAASGFTFNTYAMNWVRQAPGKGLEWVARIRSKYNNYATYYADSVKDRFTISRDDSKNTAYLQMNNLKTEDTAVYYCVRHGNFGNSYVSWFAYWGQGTLVTVSSASTKGPSVFPLAPSSKSTSGGTAALGCLVKDYFPEPVTVSWNSGALTSGVHTFPAVLQSSGLYSLSSVVTVPSSSLGTQTYICNVNHKPSNTKVDKKVEPKSCDKTHTCPPCPAPEAAGGPSVFLFPPKPKDTLMISRTPEVTCVVVDVSHEDPEVKFNWYVDGVEVHNAKTKPREEQYNSTYRVVSVLTVLHQDWLNGKEYKCKVSNKALPAPIEKTISKAKGQPREPQVYTLPPSREEMTKNQVSLYCLVKGFYPSDIAVEWESNGQPENNYKTTPPVLDSDGSFFLYSKLTVDKSRWQQGNVFSCSVMHEALHNHYTQKSLSLSPGK

SEQ ID NO: 2 - protein, 244 aa, Homo sapiens
MEFGLSWLFLVAILKGVQCEVQLVESGGGLVQPGRSLRLSCAASGFTFNDYAMHWVRQAPGKGLEWVSTISWNSGSIGYADSVKGRFTISRDNAKKSLYLQMNSLRAEDTALYYCAKDIQYGNYYYGMDVWGQGTTVTVSSASTKGPSVFPLAPSSKSTSGGTAALGCLVKDYFPEPVTVSWNSGALTSGVHTFPAVLQSSGLYSLSSVVTVPSSSLGTQTYICNVNHKPSNTKVDKKVEPKSC

SEQ ID NO: 3 - protein, 235 aa, Artificial Sequence
  humanized murine immunoglobulin light chain
MTWTPLLFLTLLLHCTGSLSELVVTQEPSLTVSPGGTVTLTCRSSTGAVTTSNYANWVQQKPGQAPRGLIGGTNKRAPGTPARFSGSLLGGKAALTLSGVQPEDEAEYYCALWYSNLWVFGGGTKLTVLGQPKAAPSVTLFPPSSEELQANKATLVCLISDFYPGAVTVAWKADSSPVKAGVETTTPSKQSNNKYAASSYLSLTPEQWKSHRSYSCQVTHEGSTVEKTVAPTECS

SEQ ID NO: 4 - protein, 253 aa, Artificial Sequence
  modified human immunoglobulin hinge and constant regions
MDMRVPAQLLGLLLLWFPGSRCPKSCDKTHTCPPCPAPEAAGGPSVFLFPPKPKDTLMISRTPEVTCVVVDVSHEDPEVKFNWYVDGVEVHNAKTKPREEQYNSTYRVVSVLTVLHQDWLNGKEYKCKVSNKALPAPIEKTISKAKGQPREPQVYTLPPSREEMTKNQVSLTCLVKGFYPSDIAVEWESNGQPENNYKTTPPVLDSDGSFFLTSKLTVDKSRWQQGNVFSCSVMHEALHNHYTQKSLSLSPGK

SEQ ID NO: 5 - protein, 691 aa, Artificial Sequence
  hybrid immunoglobulin heavy chain
MDMRVPAQLLGLLLLWFPGSRCEIVLTQSPATLSLSPGERATLSCRASQSVSSYLAWYQQKPGQAPRLLIYDASNRATGIPARFSGSGSGTDFTLTISSLEPEDFAVYYCQQRSNWPITFGQGTRLEIKRTVAAPSVFIFPPSDEQLKSGTASVVCLLNNFYPREAKVQWKVDNALQSGNSQESVTEQDSKDSTYSLSSTLTLSKADYEKHKVYACEVTHQGLSSPVTKSFNRGECEVQLLESGGGLVQPGGSLKLSCAASGFTFNTYAMNWVRQAPGKGLEWVARIRSKYNNYATYYADSVKDRFTISRDDSKNTAYLQMNNLKTEDTAVYYCVRHGNFGNSYVSWFAYWGQGTLVTVSSASTKGPSVFPLAPSSKSTSGGTAALGCLVKDYFPEPVTVSWNSGALTSGVHTFPAVLQSSGLYSLSSVVTVPSSSLGTQTYICNVNHKPSNTKVDKKVEPKSCDKTHTCPPCPAPEAAGGPSVFLFPPKPKDTLMISRTPEVTCVVVDVSHEDPEVKFNWYVDGVEVHNAKTKPREEQYNSTYRVVSVLTVLHQDWLNGKEYKCKVSNKALPAPIEKTISKAKGQPREPQVYTLPPCREEMTKNQVSLWCLVKGFYPSDIAVEWESNGQPENNYKTTPPVLDSDGSFFLYSKLTVDKSRWQQGNVFSCSVMHEALHNHYTQKSLSLSPGK

SEQ ID NO: 6 - protein, 244 aa, Homo sapiens; identical to SEQ ID NO: 2

SEQ ID NO: 7 - protein, 235 aa, Artificial Sequence; identical to SEQ ID NO: 3
  humanized immunoglobulin light chain

SEQ ID NO: 8 - protein, 253 aa, Artificial Sequence
  modified immunoglobulin hinge and constant regions
MDMRVPAQLLGLLLLWFPGSRCPKSCDKTHTCPPCPAPEAAGGPSVFLFPPKPKDTLMISRTPEVTCVVVDVSHEDPEVKFNWYVDGVEVHNAKTKPREEQYNSTYRVVSVLTVLHQDWLNGKEYKCKVSNKALPAPIEKTISKAKGQPREPQVCTLPPSREEMTKNQVSLSCAVKGFYPSDIAVEWESNGQPENNYKTTPPVLDSDGSFFLVSKLTVDKSRWQQGNVFSCSVMHEALHNHYTQKSLSLSPGK